European Patent Specification EP 3 802 859 B1, published August 30, 2023. Title: DETECTION ASSAY FOR PROTEIN-POLYNUCLEOTIDE CONJUGATES. Applicant: AMGEN INC. The sequence listing filed with the application follows.

SEQUENCE LISTING (6 sequences)

SEQ ID NO: 1 - DNA, 21 bp, Artificial Sequence
  Synthetic polynucleotide
  modified_base (1)..(21): Positions 3, 6, 9, 12, 15, 20 LNA monomers
aaacttcatctttcttcccac

SEQ ID NO: 2 - DNA, 21 bp, Artificial Sequence
  Synthetic polynucleotide
  modified_base (1)..(21): Positions 4, 8, 11, 13, 15, 17, 20 LNA monomers
ataaaatctacagtcatagga

SEQ ID NO: 3 - DNA, 21 bp, Artificial Sequence
  Synthetic polynucleotide
  modified_base (1)..(21): Positions 3, 5, 7, 12, 14, 18, 20 LNA monomers
aaacttcatcaaacttcccac

SEQ ID NO: 4 - protein, 10 aa, Artificial Sequence
  Synthetic polypeptide
EQKLISEEDL

SEQ ID NO: 5 - protein, 9 aa, Artificial Sequence
  Synthetic polypeptide
YPYDVPDYA

SEQ ID NO: 6 - protein, 8 aa, Artificial Sequence
  Synthetic polypeptide
DYKDDDDK